European Patent Application EP 4 410 811 A1, published August 7, 2024. Title: Peptide having hair loss preventing activity or hair growth promoting activity and use thereof. Applicant: CAREGENE CO., LTD. The sequence listing filed with the application follows.

SEQUENCE LISTING (17 sequences)

SEQ ID NO: 1 - protein, 10 aa, synthetic construct
QHNQIRYFEE

SEQ ID NO: 2 - DNA, 20 bp, synthetic construct
  source 1..20: mol_type = other DNA
ccagctattgtaacacctca

SEQ ID NO: 3 - DNA, 20 bp, synthetic construct
  source 1..20: mol_type = other DNA
ttcagatgtaggcagctgtc

SEQ ID NO: 4 - DNA, 25 bp, synthetic construct
  source 1..25: mol_type = other DNA
accagcagcgactctgaggaggaac

SEQ ID NO: 5 - DNA, 26 bp, synthetic construct
  source 1..26: mol_type = other DNA
tgaccctcttggcagcaggatagtcc

SEQ ID NO: 6 - DNA, 28 bp, synthetic construct
  source 1..28: mol_type = other DNA
accttcgttgccctctgtgccacagatg

SEQ ID NO: 7 - DNA, 21 bp, synthetic construct
  source 1..21: mol_type = other DNA
aggcccggaggcagtccgggt

SEQ ID NO: 8 - DNA, 20 bp, synthetic construct
  source 1..20: mol_type = other DNA
ggagccaaaagggtcatcat

SEQ ID NO: 9 - DNA, 20 bp, synthetic construct
  source 1..20: mol_type = other DNA
gtgatggcatggactgtggt

SEQ ID NO: 10 - DNA, 20 bp, synthetic construct
  source 1..20: mol_type = other DNA
gatcatcgagctgagacgca

SEQ ID NO: 11 - DNA, 20 bp, synthetic construct
  source 1..20: mol_type = other DNA
ctggccccagggtatctagt

SEQ ID NO: 12 - DNA, 20 bp, synthetic construct
  source 1..20: mol_type = other DNA
ccaaatccgcaccaaggtca

SEQ ID NO: 13 - DNA, 21 bp, synthetic construct
  source 1..21: mol_type = other DNA
gtattgattgccaggaggggg

SEQ ID NO: 14 - DNA, 20 bp, synthetic construct
  source 1..20: mol_type = other DNA
cgcggcgtatccgtgtcctc

SEQ ID NO: 15 - DNA, 24 bp, synthetic construct
  source 1..24: mol_type = other DNA
agcctgttccgtctcaaacttggt

SEQ ID NO: 16 - DNA, 20 bp, synthetic construct
  source 1..20: mol_type = other DNA
cggtcaagtcggaaaattca

SEQ ID NO: 17 - DNA, 20 bp, synthetic construct
  source 1..20: mol_type = other DNA
gaggagctgggatgtggtaa